European Patent Application EP 4 332 228 A1, published March 6, 2024. Title: Attenuated salmonella gallinarum and use thereof. Applicant: ChoyBiolab Co., Ltd INDUSTRY FOUNDATION OF CHONNAM NATIONAL UNIVERSITY. The sequence listing filed with the application follows.

SEQUENCE LISTING (10 sequences)

SEQ ID NO: 1 - DNA, 70 bp, Artificial Sequence
  rel A::kanR (Forward)
gtggatcgcaagcctgggaatttccagccagcagtcgtgtgagcgcttaggtgtaggctggagctgcttc

SEQ ID NO: 2 - DNA, 70 bp, Artificial Sequence
  rel A::kanR (Reverse)
gtgcagtcgccgtgcatcaatcacatccggcacctggttcagcttaccgaattccggggatccgtcgacc

SEQ ID NO: 3 - DNA, 69 bp, Artificial Sequence
  spot::cmR (Forward)
ttaagcgtcttcggcaggcgtatctcgttgcacgtgacgctcacgagggctgtaggctggagctgcttc

SEQ ID NO: 4 - DNA, 70 bp, Artificial Sequence
  spot::cmR (Reverse)
gccagatgtacgcgatcgcgtgcggtaaggcgaataaaggtactatagaccatatgaatatcctccttag

SEQ ID NO: 5 - DNA, 60 bp, Artificial Sequence
  ssrAB::kanR (Forward)
atgaatttgctcaatctcaagaatacgctgcaaacatcttgtgtaggctggagctgcttc

SEQ ID NO: 6 - DNA, 60 bp, Artificial Sequence
  ssrAB::kanR (Reverse)
ttaatactctattaacctcattcttcgggcacagttaagtattccggggatccgtcgacc

SEQ ID NO: 7 - DNA, 70 bp, Artificial Sequence
  Gifsy 2 prophage::cmR (Forward)
tataaatttaatatactaaccagtaaccatatcagttatgacagacaggcgtgtaggctggagctgcttc

SEQ ID NO: 8 - DNA, 84 bp, Artificial Sequence
  Gifsy 2 prophage::cmR (Reverse)
agaacacagagaaaatgtcattgcatatggtcaaaaaatagacatatttaggtccatatgaatatcctccttagttcctattcc

SEQ ID NO: 9 - DNA, 32 bp, Artificial Sequence
  glmS (Forward)
acgcggtcgacatgtgtggaattgttggcgct

SEQ ID NO: 10 - DNA, 36 bp, Artificial Sequence
  glmS (Reverse)
acgcggtcgacttactctacggtaaccgatttcgcc